European Patent Application EP 4 353 734 A1, published April 17, 2024. Title: Purification method of antibody composition. Applicant: CHIOME Bioscience Inc. The sequence listing filed with the application follows.

SEQUENCE LISTING (78 sequences)

SEQ ID NO: 1 - DNA, 420 bp, Artificial
  Recombinant DNA
  CDS (1)..(420)
atgggttggagctgtatcatcttctttctggtagcaacagctacaggcgtgcactcccaagtccagctggtgcagtctggggctgaagtgaagaagcctggggcctcagtgaaagtctcctgcaaggcttccggctacacattcactgattatgctatgcactgggtgcgacaggcccctggacaaggcctggagtggattggagttattagtacttactatggtaatacaaactacaaccagaagtttaagggcaaggccacaatgactgtcgacacatccaccagcacagcctatatggaacttaggagcttgagatctgacgatactgccgtgtattactgtgcaagaggaggattgcgagagtattactatgctatggactactggggtcaaggaaccatggtcaccgtctcctca

SEQ ID NO: 2 - protein, 140 aa, Artificial
  Synthetic Construct
MGWSCIIFFLVATATGVHSQVQLVQSGAEVKKPGASVKVSCKASGYTFTDYAMHWVRQAPGQGLEWIGVISTYYGNTNYNQKFKGKATMTVDTSTSTAYMELRSLRSDDTAVYYCARGGLREYYYAMDYWGQGTMVTVSS

SEQ ID NO: 3 - DNA, 363 bp, Artificial
  Recombinant DNA
  CDS (1)..(363)
caagtccagctggtgcagtctggggctgaagtgaagaagcctggggcctcagtgaaagtctcctgcaaggcttccggctacacattcactgattatgctatgcactgggtgcgacaggcccctggacaaggcctggagtggattggagttattagtacttactatggtaatacaaactacaaccagaagtttaagggcaaggccacaatgactgtcgacacatccaccagcacagcctatatggaacttaggagcttgagatctgacgatactgccgtgtattactgtgcaagaggaggattgcgagagtattactatgctatggactactggggtcaaggaaccatggtcaccgtctcctca

SEQ ID NO: 4 - protein, 121 aa, Artificial
  Synthetic Construct
QVQLVQSGAEVKKPGASVKVSCKASGYTFTDYAMHWVRQAPGQGLEWIGVISTYYGNTNYNQKFKGKATMTVDTSTSTAYMELRSLRSDDTAVYYCARGGLREYYYAMDYWGQGTMVTVSS

SEQ ID NO: 5 - DNA, 420 bp, Artificial
  Recombinant DNA
  CDS (1)..(420)
atgggttggagctgtatcatcttctttctggtagcaacagctacaggcgtgcactcccaagtccagctggtgcagtctggggctgaagtgaagaagcctggggcctcagtgaaagtctcctgcaaggcttccggctacacattcactgattatgctatgcactgggtgcgacaggcccctggacaaggcctggagtggattggagttattagtacttactatggtaatacaaactacaaccagaagtttaagggccgagccacaatgactgtcgacacatccaccagcacagcctatatggaacttaggagcttgagatctgacgatactgccgtgtattactgtgcaagaggaggattgcgagagtattactatgctatggactactggggtcaaggaaccatggtcaccgtctcctca

SEQ ID NO: 6 - protein, 140 aa, Artificial
  Synthetic Construct
MGWSCIIFFLVATATGVHSQVQLVQSGAEVKKPGASVKVSCKASGYTFTDYAMHWVRQAPGQGLEWIGVISTYYGNTNYNQKFKGRATMTVDTSTSTAYMELRSLRSDDTAVYYCARGGLREYYYAMDYWGQGTMVTVSS

SEQ ID NO: 7 - DNA, 363 bp, Artificial
  Recombinant DNA
  CDS (1)..(363)
caagtccagctggtgcagtctggggctgaagtgaagaagcctggggcctcagtgaaagtctcctgcaaggcttccggctacacattcactgattatgctatgcactgggtgcgacaggcccctggacaaggcctggagtggattggagttattagtacttactatggtaatacaaactacaaccagaagtttaagggccgagccacaatgactgtcgacacatccaccagcacagcctatatggaacttaggagcttgagatctgacgatactgccgtgtattactgtgcaagaggaggattgcgagagtattactatgctatggactactggggtcaaggaaccatggtcaccgtctcctca

SEQ ID NO: 8 - protein, 121 aa, Artificial
  Synthetic Construct
QVQLVQSGAEVKKPGASVKVSCKASGYTFTDYAMHWVRQAPGQGLEWIGVISTYYGNTNYNQKFKGRATMTVDTSTSTAYMELRSLRSDDTAVYYCARGGLREYYYAMDYWGQGTMVTVSS

SEQ ID NO: 9 - DNA, 399 bp, Artificial
  Recombinant DNA
  CDS (1)..(399)
atggaatcacagacccaggtcctcatgtttcttctgctctgggtatctggtgcctgtgcagacattgtcatgacacagtctccagactccctggctgtgtcactgggagagagggccactatcaactgcaagtccagtcagagccttctgaatagtagcaatcaaaagaactatttggcctggtaccagcagaaaccaggacagcctcctaaacttctggtctactttgcatccactagggaatctggggtccctgatcgcttcagtggcagtggatctgggacagatttcactcttaccatcagcagtctgcaggctgaagatgtggcagtttactactgtcagcaacattatagcactcctcccacattcggtcaggggaccaagctggagatcaaa

SEQ ID NO: 10 - protein, 133 aa, Artificial
  Synthetic Construct
MESQTQVLMFLLLWVSGACADIVMTQSPDSLAVSLGERATINCKSSQSLLNSSNQKNYLAWYQQKPGQPPKLLVYFASTRESGVPDRFSGSGSGTDFTLTISSLQAEDVAVYYCQQHYSTPPTFGQGTKLEIK

SEQ ID NO: 11 - DNA, 339 bp, Artificial
  Recombinant DNA
  CDS (1)..(339)
gacattgtcatgacacagtctccagactccctggctgtgtcactgggagagagggccactatcaactgcaagtccagtcagagccttctgaatagtagcaatcaaaagaactatttggcctggtaccagcagaaaccaggacagcctcctaaacttctggtctactttgcatccactagggaatctggggtccctgatcgcttcagtggcagtggatctgggacagatttcactcttaccatcagcagtctgcaggctgaagatgtggcagtttactactgtcagcaacattatagcactcctcccacattcggtcaggggaccaagctggagatcaaa

SEQ ID NO: 12 - protein, 113 aa, Artificial
  Synthetic Construct
DIVMTQSPDSLAVSLGERATINCKSSQSLLNSSNQKNYLAWYQQKPGQPPKLLVYFASTRESGVPDRFSGSGSGTDFTLTISSLQAEDVAVYYCQQHYSTPPTFGQGTKLEIK

SEQ ID NO: 13 - DNA, 420 bp, Artificial
  Recombinant DNA
  CDS (1)..(420)
atgggttggagctgtatcatcttctttctggtagcaacagctacaggcgtgcactcccaagtccagctggtgcagtctggggctgaagtgaagaagcctggggcctcagtgaaagtctcctgcaagggttccggctacacattcactgattatgctatgcactgggtgcgacaggcccctggacaaggcctggagtggattggagttattagtacttactatggtaatacaaactacaaccagaagtttaagggcaaggccacaatgactgtcgacacatccaccagcacagcctatatggaacttaggagcttgagatctgacgatactgccgtgtattactgtgcaagaggaggattgcgagagtattactatgctatggactactggggtcaaggaaccatggtcaccgtctcctca

SEQ ID NO: 14 - protein, 140 aa, Artificial
  Synthetic Construct
MGWSCIIFFLVATATGVHSQVQLVQSGAEVKKPGASVKVSCKGSGYTFTDYAMHWVRQAPGQGLEWIGVISTYYGNTNYNQKFKGKATMTVDTSTSTAYMELRSLRSDDTAVYYCARGGLREYYYAMDYWGQGTMVTVSS

SEQ ID NO: 15 - DNA, 363 bp, Artificial
  Recombinant DNA
  CDS (1)..(363)
caagtccagctggtgcagtctggggctgaagtgaagaagcctggggcctcagtgaaagtctcctgcaagggttccggctacacattcactgattatgctatgcactgggtgcgacaggcccctggacaaggcctggagtggattggagttattagtacttactatggtaatacaaactacaaccagaagtttaagggcaaggccacaatgactgtcgacacatccaccagcacagcctatatggaacttaggagcttgagatctgacgatactgccgtgtattactgtgcaagaggaggattgcgagagtattactatgctatggactactggggtcaaggaaccatggtcaccgtctcctca

SEQ ID NO: 16 - protein, 121 aa, Artificial
  Synthetic Construct
QVQLVQSGAEVKKPGASVKVSCKGSGYTFTDYAMHWVRQAPGQGLEWIGVISTYYGNTNYNQKFKGKATMTVDTSTSTAYMELRSLRSDDTAVYYCARGGLREYYYAMDYWGQGTMVTVSS

SEQ ID NO: 17 - DNA, 420 bp, Artificial
  Recombinant DNA
  CDS (1)..(420)
atgggttggagctgtatcatcttctttctggtagcaacagctacaggcgtgcactcccaagtccagctggtgcagtctggggctgaagtgaagaagcctggggcctcagtgaaagtctcctgcaaggcttccggctacacattcactgattatgctatgcactgggtgcgacaggcccctggacaaggcctggagtggattggagttattagtacttactatggtaatacaaactacaaccagaagtttaagggcaaggccacaatgactgtcgacaaatccaccagcacagcctatatggaacttaggagcttgagatctgacgatactgccgtgtattactgtgcaagaggaggattgcgagagtattactatgctatggactactggggtcaaggaaccatggtcaccgtctcctca

SEQ ID NO: 18 - protein, 140 aa, Artificial
  Synthetic Construct
MGWSCIIFFLVATATGVHSQVQLVQSGAEVKKPGASVKVSCKASGYTFTDYAMHWVRQAPGQGLEWIGVISTYYGNTNYNQKFKGKATMTVDKSTSTAYMELRSLRSDDTAVYYCARGGLREYYYAMDYWGQGTMVTVSS

SEQ ID NO: 19 - DNA, 363 bp, Artificial
  Recombinant DNA
  CDS (1)..(363)
caagtccagctggtgcagtctggggctgaagtgaagaagcctggggcctcagtgaaagtctcctgcaaggcttccggctacacattcactgattatgctatgcactgggtgcgacaggcccctggacaaggcctggagtggattggagttattagtacttactatggtaatacaaactacaaccagaagtttaagggcaaggccacaatgactgtcgacaaatccaccagcacagcctatatggaacttaggagcttgagatctgacgatactgccgtgtattactgtgcaagaggaggattgcgagagtattactatgctatggactactggggtcaaggaaccatggtcaccgtctcctca

SEQ ID NO: 20 - protein, 121 aa, Artificial
  Synthetic Construct
QVQLVQSGAEVKKPGASVKVSCKASGYTFTDYAMHWVRQAPGQGLEWIGVISTYYGNTNYNQKFKGKATMTVDKSTSTAYMELRSLRSDDTAVYYCARGGLREYYYAMDYWGQGTMVTVSS

SEQ ID NO: 21 - DNA, 420 bp, Artificial
  Recombinant DNA
  CDS (1)..(420)
atgggttggagctgtatcatcttctttctggtagcaacagctacaggcgtgcactcccaagtccagctggtgcagtctggggctgaagtgaagaagcctggggcctcagtgaaagtctcctgcaagggttccggctacacattcactgattatgctatgcactgggtgcgacaggcccctggacaaggcctggagtggattggagttattagtacttactatggtaatacaaactacaaccagaagtttaagggcaaggccacaatgactgtcgacaaatccaccagcacagcctatatggaacttaggagcttgagatctgacgatactgccgtgtattactgtgcaagaggaggattgcgagagtattactatgctatggactactggggtcaaggaaccatggtcaccgtctcctca

SEQ ID NO: 22 - protein, 140 aa, Artificial
  Synthetic Construct
MGWSCIIFFLVATATGVHSQVQLVQSGAEVKKPGASVKVSCKGSGYTFTDYAMHWVRQAPGQGLEWIGVISTYYGNTNYNQKFKGKATMTVDKSTSTAYMELRSLRSDDTAVYYCARGGLREYYYAMDYWGQGTMVTVSS

SEQ ID NO: 23 - DNA, 363 bp, Artificial
  Recombinant DNA
  CDS (1)..(363)
caagtccagctggtgcagtctggggctgaagtgaagaagcctggggcctcagtgaaagtctcctgcaagggttccggctacacattcactgattatgctatgcactgggtgcgacaggcccctggacaaggcctggagtggattggagttattagtacttactatggtaatacaaactacaaccagaagtttaagggcaaggccacaatgactgtcgacaaatccaccagcacagcctatatggaacttaggagcttgagatctgacgatactgccgtgtattactgtgcaagaggaggattgcgagagtattactatgctatggactactggggtcaaggaaccatggtcaccgtctcctca

SEQ ID NO: 24 - protein, 121 aa, Artificial
  Synthetic Construct
QVQLVQSGAEVKKPGASVKVSCKGSGYTFTDYAMHWVRQAPGQGLEWIGVISTYYGNTNYNQKFKGKATMTVDKSTSTAYMELRSLRSDDTAVYYCARGGLREYYYAMDYWGQGTMVTVSS

SEQ ID NO: 25 - DNA, 420 bp, Artificial
  Recombinant DNA
  CDS (1)..(420)
atgggttggagctgtatcatcttctttctggtagcaacagctacaggcgtgcactcccaagtccagctggtgcagtctggggctgaagtgaagaagcctggggcctcagtgaaagtctcctgcaagggttccggctacacattcactgattatgctatgcactgggtgcgacaggcccctggacaaggcctggagtggattggagttattagtacttactatggtaatacaaactacaaccagaagtttaagggccgagccacaatgactgtcgacacatccaccagcacagcctatatggaacttaggagcttgagatctgacgatactgccgtgtattactgtgcaagaggaggattgcgagagtattactatgctatggactactggggtcaaggaaccatggtcaccgtctcctca

SEQ ID NO: 26 - protein, 140 aa, Artificial
  Synthetic Construct
MGWSCIIFFLVATATGVHSQVQLVQSGAEVKKPGASVKVSCKGSGYTFTDYAMHWVRQAPGQGLEWIGVISTYYGNTNYNQKFKGRATMTVDTSTSTAYMELRSLRSDDTAVYYCARGGLREYYYAMDYWGQGTMVTVSS

SEQ ID NO: 27 - DNA, 363 bp, Artificial
  Recombinant DNA
  CDS (1)..(363)
caagtccagctggtgcagtctggggctgaagtgaagaagcctggggcctcagtgaaagtctcctgcaagggttccggctacacattcactgattatgctatgcactgggtgcgacaggcccctggacaaggcctggagtggattggagttattagtacttactatggtaatacaaactacaaccagaagtttaagggccgagccacaatgactgtcgacacatccaccagcacagcctatatggaacttaggagcttgagatctgacgatactgccgtgtattactgtgcaagaggaggattgcgagagtattactatgctatggactactggggtcaaggaaccatggtcaccgtctcctca

SEQ ID NO: 28 - protein, 121 aa, Artificial
  Synthetic Construct
QVQLVQSGAEVKKPGASVKVSCKGSGYTFTDYAMHWVRQAPGQGLEWIGVISTYYGNTNYNQKFKGRATMTVDTSTSTAYMELRSLRSDDTAVYYCARGGLREYYYAMDYWGQGTMVTVSS

SEQ ID NO: 29 - DNA, 420 bp, Artificial
  Recombinant DNA
  CDS (1)..(420)
atgggttggagctgtatcatcttctttctggtagcaacagctacaggcgtgcactcccaagtccagctggtgcagtctggggctgaagtgaagaagcctggggcctcagtgaaagtctcctgcaaggcttccggctacacattcactgattatgctatgcactgggtgcgacaggcccctggacaaggcctggagtggattggagttattagtacttactatggtaatacaaactacaaccagaagtttaagggccgagccacaatgactgtcgacaaatccaccagcacagcctatatggaacttaggagcttgagatctgacgatactgccgtgtattactgtgcaagaggaggattgcgagagtattactatgctatggactactggggtcaaggaaccatggtcaccgtctcctca

SEQ ID NO: 30 - protein, 140 aa, Artificial
  Synthetic Construct
MGWSCIIFFLVATATGVHSQVQLVQSGAEVKKPGASVKVSCKASGYTFTDYAMHWVRQAPGQGLEWIGVISTYYGNTNYNQKFKGRATMTVDKSTSTAYMELRSLRSDDTAVYYCARGGLREYYYAMDYWGQGTMVTVSS

SEQ ID NO: 31 - DNA, 363 bp, Artificial
  Recombinant DNA
  CDS (1)..(363)
caagtccagctggtgcagtctggggctgaagtgaagaagcctggggcctcagtgaaagtctcctgcaaggcttccggctacacattcactgattatgctatgcactgggtgcgacaggcccctggacaaggcctggagtggattggagttattagtacttactatggtaatacaaactacaaccagaagtttaagggccgagccacaatgactgtcgacaaatccaccagcacagcctatatggaacttaggagcttgagatctgacgatactgccgtgtattactgtgcaagaggaggattgcgagagtattactatgctatggactactggggtcaaggaaccatggtcaccgtctcctca

SEQ ID NO: 32 - protein, 121 aa, Artificial
  Synthetic Construct
QVQLVQSGAEVKKPGASVKVSCKASGYTFTDYAMHWVRQAPGQGLEWIGVISTYYGNTNYNQKFKGRATMTVDKSTSTAYMELRSLRSDDTAVYYCARGGLREYYYAMDYWGQGTMVTVSS

SEQ ID NO: 33 - DNA, 420 bp, Artificial
  Recombinant DNA
  CDS (1)..(420)
atgggttggagctgtatcatcttctttctggtagcaacagctacaggcgtgcactcccaagtccagctggtgcagtctggggctgaagtgaagaagcctggggcctcagtgaaagtctcctgcaagggttccggctacacattcactgattatgctatgcactgggtgcgacaggcccctggacaaggcctggagtggattggagttattagtacttactatggtaatacaaactacaaccagaagtttaagggccgagccacaatgactgtcgacaaatccaccagcacagcctatatggaacttaggagcttgagatctgacgatactgccgtgtattactgtgcaagaggaggattgcgagagtattactatgctatggactactggggtcaaggaaccatggtcaccgtctcctca

SEQ ID NO: 34 - protein, 140 aa, Artificial
  Synthetic Construct
MGWSCIIFFLVATATGVHSQVQLVQSGAEVKKPGASVKVSCKGSGYTFTDYAMHWVRQAPGQGLEWIGVISTYYGNTNYNQKFKGRATMTVDKSTSTAYMELRSLRSDDTAVYYCARGGLREYYYAMDYWGQGTMVTVSS

SEQ ID NO: 35 - DNA, 363 bp, Artificial
  Recombinant DNA
  CDS (1)..(363)
caagtccagctggtgcagtctggggctgaagtgaagaagcctggggcctcagtgaaagtctcctgcaagggttccggctacacattcactgattatgctatgcactgggtgcgacaggcccctggacaaggcctggagtggattggagttattagtacttactatggtaatacaaactacaaccagaagtttaagggccgagccacaatgactgtcgacaaatccaccagcacagcctatatggaacttaggagcttgagatctgacgatactgccgtgtattactgtgcaagaggaggattgcgagagtattactatgctatggactactggggtcaaggaaccatggtcaccgtctcctca

SEQ ID NO: 36 - protein, 121 aa, Artificial
  Synthetic Construct
QVQLVQSGAEVKKPGASVKVSCKGSGYTFTDYAMHWVRQAPGQGLEWIGVISTYYGNTNYNQKFKGRATMTVDKSTSTAYMELRSLRSDDTAVYYCARGGLREYYYAMDYWGQGTMVTVSS

SEQ ID NO: 37 - DNA, 1413 bp, Artificial Sequence
  antibody
  CDS (1)..(1413)
atgggttggagctgtatcatcttctttctggtagcaacagctacaggcgtgcactcccaagtccagctggtgcagtctggggctgaagtgaagaagcctggggcctcagtgaaagtctcctgcaaggcttccggctacacattcactgattatgctatgcactgggtgcgacaggcccctggacaaggcctggagtggattggagttattagtacttactatggtaatacaaactacaaccagaagtttaagggcaaggccacaatgactgtcgacacatccaccagcacagcctatatggaacttaggagcttgagatctgacgatactgccgtgtattactgtgcaagaggaggattgcgagagtattactatgctatggactactggggtcaaggaaccatggtcaccgtctcctcagcctccaccaagggcccatcggtcttccccctggcaccctcctccaagagcacctctgggggcacagcggccctgggctgcctggtcaaggactacttccccgaaccggtgacggtgtcgtggaactcaggcgccctgaccagcggcgtgcacaccttcccggctgtcctacagtcctcaggactctactccctcagcagcgtggtgaccgtgccctccagcagcttgggcacccagacctacatctgcaacgtgaatcacaagcccagcaacaccaaggtggacaagaaagttgagcccaaatcttgtgacaaaactcacacatgcccaccgtgcccagcacctgaactcctggggggaccgtcagtcttcctcttccccccaaaacccaaggacaccctcatgatctcccggacccctgaggtcacatgcgtggtggtggacgtgagccacgaagaccctgaggtcaagttcaactggtacgtggacggcgtggaggtgcataatgccaagacaaagccgcgggaggagcagtacaacagcacgtaccgtgtggtcagcgtcctcaccgtcctgcaccaggactggctgaatggcaaggagtacaagtgcaaggtctccaacaaagccctcccagcccccatcgagaaaaccatctccaaagccaaagggcagccccgagaaccacaggtgtacaccctgcccccatcccgggatgagctgaccaagaaccaggtcagcctgacctgcctggtcaaaggcttctatcccagcgacatcgccgtggagtgggagagcaatgggcagccggagaacaactacaagaccacgcctcccgtgctggactccgacggctccttcttcctctacagcaagctcaccgtggacaagagcaggtggcagcaggggaacgtcttctcatgctccgtgatgcatgaggctctgcacaaccactacacgcagaagagcctctccctgtctccgggtaaatga

SEQ ID NO: 38 - protein, 470 aa, Artificial Sequence
  Synthetic Construct
MGWSCIIFFLVATATGVHSQVQLVQSGAEVKKPGASVKVSCKASGYTFTDYAMHWVRQAPGQGLEWIGVISTYYGNTNYNQKFKGKATMTVDTSTSTAYMELRSLRSDDTAVYYCARGGLREYYYAMDYWGQGTMVTVSSASTKGPSVFPLAPSSKSTSGGTAALGCLVKDYFPEPVTVSWNSGALTSGVHTFPAVLQSSGLYSLSSVVTVPSSSLGTQTYICNVNHKPSNTKVDKKVEPKSCDKTHTCPPCPAPELLGGPSVFLFPPKPKDTLMISRTPEVTCVVVDVSHEDPEVKFNWYVDGVEVHNAKTKPREEQYNSTYRVVSVLTVLHQDWLNGKEYKCKVSNKALPAPIEKTISKAKGQPREPQVYTLPPSRDELTKNQVSLTCLVKGFYPSDIAVEWESNGQPENNYKTTPPVLDSDGSFFLYSKLTVDKSRWQQGNVFSCSVMHEALHNHYTQKSLSLSPGK

SEQ ID NO: 39 - DNA, 1356 bp, Artificial Sequence
  antibody
  CDS (1)..(1356)
caagtccagctggtgcagtctggggctgaagtgaagaagcctggggcctcagtgaaagtctcctgcaaggcttccggctacacattcactgattatgctatgcactgggtgcgacaggcccctggacaaggcctggagtggattggagttattagtacttactatggtaatacaaactacaaccagaagtttaagggcaaggccacaatgactgtcgacacatccaccagcacagcctatatggaacttaggagcttgagatctgacgatactgccgtgtattactgtgcaagaggaggattgcgagagtattactatgctatggactactggggtcaaggaaccatggtcaccgtctcctcagcctccaccaagggcccatcggtcttccccctggcaccctcctccaagagcacctctgggggcacagcggccctgggctgcctggtcaaggactacttccccgaaccggtgacggtgtcgtggaactcaggcgccctgaccagcggcgtgcacaccttcccggctgtcctacagtcctcaggactctactccctcagcagcgtggtgaccgtgccctccagcagcttgggcacccagacctacatctgcaacgtgaatcacaagcccagcaacaccaaggtggacaagaaagttgagcccaaatcttgtgacaaaactcacacatgcccaccgtgcccagcacctgaactcctggggggaccgtcagtcttcctcttccccccaaaacccaaggacaccctcatgatctcccggacccctgaggtcacatgcgtggtggtggacgtgagccacgaagaccctgaggtcaagttcaactggtacgtggacggcgtggaggtgcataatgccaagacaaagccgcgggaggagcagtacaacagcacgtaccgtgtggtcagcgtcctcaccgtcctgcaccaggactggctgaatggcaaggagtacaagtgcaaggtctccaacaaagccctcccagcccccatcgagaaaaccatctccaaagccaaagggcagccccgagaaccacaggtgtacaccctgcccccatcccgggatgagctgaccaagaaccaggtcagcctgacctgcctggtcaaaggcttctatcccagcgacatcgccgtggagtgggagagcaatgggcagccggagaacaactacaagaccacgcctcccgtgctggactccgacggctccttcttcctctacagcaagctcaccgtggacaagagcaggtggcagcaggggaacgtcttctcatgctccgtgatgcatgaggctctgcacaaccactacacgcagaagagcctctccctgtctccgggtaaatga

SEQ ID NO: 40 - protein, 451 aa, Artificial Sequence
  Synthetic Construct
QVQLVQSGAEVKKPGASVKVSCKASGYTFTDYAMHWVRQAPGQGLEWIGVISTYYGNTNYNQKFKGKATMTVDTSTSTAYMELRSLRSDDTAVYYCARGGLREYYYAMDYWGQGTMVTVSSASTKGPSVFPLAPSSKSTSGGTAALGCLVKDYFPEPVTVSWNSGALTSGVHTFPAVLQSSGLYSLSSVVTVPSSSLGTQTYICNVNHKPSNTKVDKKVEPKSCDKTHTCPPCPAPELLGGPSVFLFPPKPKDTLMISRTPEVTCVVVDVSHEDPEVKFNWYVDGVEVHNAKTKPREEQYNSTYRVVSVLTVLHQDWLNGKEYKCKVSNKALPAPIEKTISKAKGQPREPQVYTLPPSRDELTKNQVSLTCLVKGFYPSDIAVEWESNGQPENNYKTTPPVLDSDGSFFLYSKLTVDKSRWQQGNVFSCSVMHEALHNHYTQKSLSLSPGK

SEQ ID NO: 41 - DNA, 1413 bp, Artificial Sequence
  antibody
  CDS (1)..(1413)
atgggttggagctgtatcatcttctttctggtagcaacagctacaggcgtgcactcccaagtccagctggtgcagtctggggctgaagtgaagaagcctggggcctcagtgaaagtctcctgcaaggcttccggctacacattcactgattatgctatgcactgggtgcgacaggcccctggacaaggcctggagtggattggagttattagtacttactatggtaatacaaactacaaccagaagtttaagggccgagccacaatgactgtcgacacatccaccagcacagcctatatggaacttaggagcttgagatctgacgatactgccgtgtattactgtgcaagaggaggattgcgagagtattactatgctatggactactggggtcaaggaaccatggtcaccgtctcctcagcctccaccaagggcccatcggtcttccccctggcaccctcctccaagagcacctctgggggcacagcggccctgggctgcctggtcaaggactacttccccgaaccggtgacggtgtcgtggaactcaggcgccctgaccagcggcgtgcacaccttcccggctgtcctacagtcctcaggactctactccctcagcagcgtggtgaccgtgccctccagcagcttgggcacccagacctacatctgcaacgtgaatcacaagcccagcaacaccaaggtggacaagaaagttgagcccaaatcttgtgacaaaactcacacatgcccaccgtgcccagcacctgaactcctggggggaccgtcagtcttcctcttccccccaaaacccaaggacaccctcatgatctcccggacccctgaggtcacatgcgtggtggtggacgtgagccacgaagaccctgaggtcaagttcaactggtacgtggacggcgtggaggtgcataatgccaagacaaagccgcgggaggagcagtacaacagcacgtaccgtgtggtcagcgtcctcaccgtcctgcaccaggactggctgaatggcaaggagtacaagtgcaaggtctccaacaaagccctcccagcccccatcgagaaaaccatctccaaagccaaagggcagccccgagaaccacaggtgtacaccctgcccccatcccgggatgagctgaccaagaaccaggtcagcctgacctgcctggtcaaaggcttctatcccagcgacatcgccgtggagtgggagagcaatgggcagccggagaacaactacaagaccacgcctcccgtgctggactccgacggctccttcttcctctacagcaagctcaccgtggacaagagcaggtggcagcaggggaacgtcttctcatgctccgtgatgcatgaggctctgcacaaccactacacgcagaagagcctctccctgtctccgggtaaatga

SEQ ID NO: 42 - protein, 470 aa, Artificial Sequence
  Synthetic Construct
MGWSCIIFFLVATATGVHSQVQLVQSGAEVKKPGASVKVSCKASGYTFTDYAMHWVRQAPGQGLEWIGVISTYYGNTNYNQKFKGRATMTVDTSTSTAYMELRSLRSDDTAVYYCARGGLREYYYAMDYWGQGTMVTVSSASTKGPSVFPLAPSSKSTSGGTAALGCLVKDYFPEPVTVSWNSGALTSGVHTFPAVLQSSGLYSLSSVVTVPSSSLGTQTYICNVNHKPSNTKVDKKVEPKSCDKTHTCPPCPAPELLGGPSVFLFPPKPKDTLMISRTPEVTCVVVDVSHEDPEVKFNWYVDGVEVHNAKTKPREEQYNSTYRVVSVLTVLHQDWLNGKEYKCKVSNKALPAPIEKTISKAKGQPREPQVYTLPPSRDELTKNQVSLTCLVKGFYPSDIAVEWESNGQPENNYKTTPPVLDSDGSFFLYSKLTVDKSRWQQGNVFSCSVMHEALHNHYTQKSLSLSPGK

SEQ ID NO: 43 - DNA, 1356 bp, Artificial Sequence
  antibody
  CDS (1)..(1356)
caagtccagctggtgcagtctggggctgaagtgaagaagcctggggcctcagtgaaagtctcctgcaaggcttccggctacacattcactgattatgctatgcactgggtgcgacaggcccctggacaaggcctggagtggattggagttattagtacttactatggtaatacaaactacaaccagaagtttaagggccgagccacaatgactgtcgacacatccaccagcacagcctatatggaacttaggagcttgagatctgacgatactgccgtgtattactgtgcaagaggaggattgcgagagtattactatgctatggactactggggtcaaggaaccatggtcaccgtctcctcagcctccaccaagggcccatcggtcttccccctggcaccctcctccaagagcacctctgggggcacagcggccctgggctgcctggtcaaggactacttccccgaaccggtgacggtgtcgtggaactcaggcgccctgaccagcggcgtgcacaccttcccggctgtcctacagtcctcaggactctactccctcagcagcgtggtgaccgtgccctccagcagcttgggcacccagacctacatctgcaacgtgaatcacaagcccagcaacaccaaggtggacaagaaagttgagcccaaatcttgtgacaaaactcacacatgcccaccgtgcccagcacctgaactcctggggggaccgtcagtcttcctcttccccccaaaacccaaggacaccctcatgatctcccggacccctgaggtcacatgcgtggtggtggacgtgagccacgaagaccctgaggtcaagttcaactggtacgtggacggcgtggaggtgcataatgccaagacaaagccgcgggaggagcagtacaacagcacgtaccgtgtggtcagcgtcctcaccgtcctgcaccaggactggctgaatggcaaggagtacaagtgcaaggtctccaacaaagccctcccagcccccatcgagaaaaccatctccaaagccaaagggcagccccgagaaccacaggtgtacaccctgcccccatcccgggatgagctgaccaagaaccaggtcagcctgacctgcctggtcaaaggcttctatcccagcgacatcgccgtggagtgggagagcaatgggcagccggagaacaactacaagaccacgcctcccgtgctggactccgacggctccttcttcctctacagcaagctcaccgtggacaagagcaggtggcagcaggggaacgtcttctcatgctccgtgatgcatgaggctctgcacaaccactacacgcagaagagcctctccctgtctccgggtaaatga

SEQ ID NO: 44 - protein, 451 aa, Artificial Sequence
  Synthetic Construct
QVQLVQSGAEVKKPGASVKVSCKASGYTFTDYAMHWVRQAPGQGLEWIGVISTYYGNTNYNQKFKGRATMTVDTSTSTAYMELRSLRSDDTAVYYCARGGLREYYYAMDYWGQGTMVTVSSASTKGPSVFPLAPSSKSTSGGTAALGCLVKDYFPEPVTVSWNSGALTSGVHTFPAVLQSSGLYSLSSVVTVPSSSLGTQTYICNVNHKPSNTKVDKKVEPKSCDKTHTCPPCPAPELLGGPSVFLFPPKPKDTLMISRTPEVTCVVVDVSHEDPEVKFNWYVDGVEVHNAKTKPREEQYNSTYRVVSVLTVLHQDWLNGKEYKCKVSNKALPAPIEKTISKAKGQPREPQVYTLPPSRDELTKNQVSLTCLVKGFYPSDIAVEWESNGQPENNYKTTPPVLDSDGSFFLYSKLTVDKSRWQQGNVFSCSVMHEALHNHYTQKSLSLSPGK

SEQ ID NO: 45 - DNA, 1413 bp, Artificial Sequence
  antibody
  CDS (1)..(1413)
atgggttggagctgtatcatcttctttctggtagcaacagctacaggcgtgcactcccaagtccagctggtgcagtctggggctgaagtgaagaagcctggggcctcagtgaaagtctcctgcaagggttccggctacacattcactgattatgctatgcactgggtgcgacaggcccctggacaaggcctggagtggattggagttattagtacttactatggtaatacaaactacaaccagaagtttaagggcaaggccacaatgactgtcgacacatccaccagcacagcctatatggaacttaggagcttgagatctgacgatactgccgtgtattactgtgcaagaggaggattgcgagagtattactatgctatggactactggggtcaaggaaccatggtcaccgtctcctcagcctccaccaagggcccatcggtcttccccctggcaccctcctccaagagcacctctgggggcacagcggccctgggctgcctggtcaaggactacttccccgaaccggtgacggtgtcgtggaactcaggcgccctgaccagcggcgtgcacaccttcccggctgtcctacagtcctcaggactctactccctcagcagcgtggtgaccgtgccctccagcagcttgggcacccagacctacatctgcaacgtgaatcacaagcccagcaacaccaaggtggacaagaaagttgagcccaaatcttgtgacaaaactcacacatgcccaccgtgcccagcacctgaactcctggggggaccgtcagtcttcctcttccccccaaaacccaaggacaccctcatgatctcccggacccctgaggtcacatgcgtggtggtggacgtgagccacgaagaccctgaggtcaagttcaactggtacgtggacggcgtggaggtgcataatgccaagacaaagccgcgggaggagcagtacaacagcacgtaccgtgtggtcagcgtcctcaccgtcctgcaccaggactggctgaatggcaaggagtacaagtgcaaggtctccaacaaagccctcccagcccccatcgagaaaaccatctccaaagccaaagggcagccccgagaaccacaggtgtacaccctgcccccatcccgggatgagctgaccaagaaccaggtcagcctgacctgcctggtcaaaggcttctatcccagcgacatcgccgtggagtgggagagcaatgggcagccggagaacaactacaagaccacgcctcccgtgctggactccgacggctccttcttcctctacagcaagctcaccgtggacaagagcaggtggcagcaggggaacgtcttctcatgctccgtgatgcatgaggctctgcacaaccactacacgcagaagagcctctccctgtctccgggtaaatga

SEQ ID NO: 46 - protein, 470 aa, Artificial Sequence
  Synthetic Construct
MGWSCIIFFLVATATGVHSQVQLVQSGAEVKKPGASVKVSCKGSGYTFTDYAMHWVRQAPGQGLEWIGVISTYYGNTNYNQKFKGKATMTVDTSTSTAYMELRSLRSDDTAVYYCARGGLREYYYAMDYWGQGTMVTVSSASTKGPSVFPLAPSSKSTSGGTAALGCLVKDYFPEPVTVSWNSGALTSGVHTFPAVLQSSGLYSLSSVVTVPSSSLGTQTYICNVNHKPSNTKVDKKVEPKSCDKTHTCPPCPAPELLGGPSVFLFPPKPKDTLMISRTPEVTCVVVDVSHEDPEVKFNWYVDGVEVHNAKTKPREEQYNSTYRVVSVLTVLHQDWLNGKEYKCKVSNKALPAPIEKTISKAKGQPREPQVYTLPPSRDELTKNQVSLTCLVKGFYPSDIAVEWESNGQPENNYKTTPPVLDSDGSFFLYSKLTVDKSRWQQGNVFSCSVMHEALHNHYTQKSLSLSPGK

SEQ ID NO: 47 - DNA, 1356 bp, Artificial Sequence
  antibody
  CDS (1)..(1356)
caagtccagctggtgcagtctggggctgaagtgaagaagcctggggcctcagtgaaagtctcctgcaagggttccggctacacattcactgattatgctatgcactgggtgcgacaggcccctggacaaggcctggagtggattggagttattagtacttactatggtaatacaaactacaaccagaagtttaagggcaaggccacaatgactgtcgacacatccaccagcacagcctatatggaacttaggagcttgagatctgacgatactgccgtgtattactgtgcaagaggaggattgcgagagtattactatgctatggactactggggtcaaggaaccatggtcaccgtctcctcagcctccaccaagggcccatcggtcttccccctggcaccctcctccaagagcacctctgggggcacagcggccctgggctgcctggtcaaggactacttccccgaaccggtgacggtgtcgtggaactcaggcgccctgaccagcggcgtgcacaccttcccggctgtcctacagtcctcaggactctactccctcagcagcgtggtgaccgtgccctccagcagcttgggcacccagacctacatctgcaacgtgaatcacaagcccagcaacaccaaggtggacaagaaagttgagcccaaatcttgtgacaaaactcacacatgcccaccgtgcccagcacctgaactcctggggggaccgtcagtcttcctcttccccccaaaacccaaggacaccctcatgatctcccggacccctgaggtcacatgcgtggtggtggacgtgagccacgaagaccctgaggtcaagttcaactggtacgtggacggcgtggaggtgcataatgccaagacaaagccgcgggaggagcagtacaacagcacgtaccgtgtggtcagcgtcctcaccgtcctgcaccaggactggctgaatggcaaggagtacaagtgcaaggtctccaacaaagccctcccagcccccatcgagaaaaccatctccaaagccaaagggcagccccgagaaccacaggtgtacaccctgcccccatcccgggatgagctgaccaagaaccaggtcagcctgacctgcctggtcaaaggcttctatcccagcgacatcgccgtggagtgggagagcaatgggcagccggagaacaactacaagaccacgcctcccgtgctggactccgacggctccttcttcctctacagcaagctcaccgtggacaagagcaggtggcagcaggggaacgtcttctcatgctccgtgatgcatgaggctctgcacaaccactacacgcagaagagcctctccctgtctccgggtaaatga

SEQ ID NO: 48 - protein, 451 aa, Artificial Sequence
  Synthetic Construct
QVQLVQSGAEVKKPGASVKVSCKGSGYTFTDYAMHWVRQAPGQGLEWIGVISTYYGNTNYNQKFKGKATMTVDTSTSTAYMELRSLRSDDTAVYYCARGGLREYYYAMDYWGQGTMVTVSSASTKGPSVFPLAPSSKSTSGGTAALGCLVKDYFPEPVTVSWNSGALTSGVHTFPAVLQSSGLYSLSSVVTVPSSSLGTQTYICNVNHKPSNTKVDKKVEPKSCDKTHTCPPCPAPELLGGPSVFLFPPKPKDTLMISRTPEVTCVVVDVSHEDPEVKFNWYVDGVEVHNAKTKPREEQYNSTYRVVSVLTVLHQDWLNGKEYKCKVSNKALPAPIEKTISKAKGQPREPQVYTLPPSRDELTKNQVSLTCLVKGFYPSDIAVEWESNGQPENNYKTTPPVLDSDGSFFLYSKLTVDKSRWQQGNVFSCSVMHEALHNHYTQKSLSLSPGK

SEQ ID NO: 49 - DNA, 1413 bp, Artificial Sequence
  antibody
  CDS (1)..(1413)
atgggttggagctgtatcatcttctttctggtagcaacagctacaggcgtgcactcccaagtccagctggtgcagtctggggctgaagtgaagaagcctggggcctcagtgaaagtctcctgcaagggttccggctacacattcactgattatgctatgcactgggtgcgacaggcccctggacaaggcctggagtggattggagttattagtacttactatggtaatacaaactacaaccagaagtttaagggccgagccacaatgactgtcgacacatccaccagcacagcctatatggaacttaggagcttgagatctgacgatactgccgtgtattactgtgcaagaggaggattgcgagagtattactatgctatggactactggggtcaaggaaccatggtcaccgtctcctcagcctccaccaagggcccatcggtcttccccctggcaccctcctccaagagcacctctgggggcacagcggccctgggctgcctggtcaaggactacttccccgaaccggtgacggtgtcgtggaactcaggcgccctgaccagcggcgtgcacaccttcccggctgtcctacagtcctcaggactctactccctcagcagcgtggtgaccgtgccctccagcagcttgggcacccagacctacatctgcaacgtgaatcacaagcccagcaacaccaaggtggacaagaaagttgagcccaaatcttgtgacaaaactcacacatgcccaccgtgcccagcacctgaactcctggggggaccgtcagtcttcctcttccccccaaaacccaaggacaccctcatgatctcccggacccctgaggtcacatgcgtggtggtggacgtgagccacgaagaccctgaggtcaagttcaactggtacgtggacggcgtggaggtgcataatgccaagacaaagccgcgggaggagcagtacaacagcacgtaccgtgtggtcagcgtcctcaccgtcctgcaccaggactggctgaatggcaaggagtacaagtgcaaggtctccaacaaagccctcccagcccccatcgagaaaaccatctccaaagccaaagggcagccccgagaaccacaggtgtacaccctgcccccatcccgggatgagctgaccaagaaccaggtcagcctgacctgcctggtcaaaggcttctatcccagcgacatcgccgtggagtgggagagcaatgggcagccggagaacaactacaagaccacgcctcccgtgctggactccgacggctccttcttcctctacagcaagctcaccgtggacaagagcaggtggcagcaggggaacgtcttctcatgctccgtgatgcatgaggctctgcacaaccactacacgcagaagagcctctccctgtctccgggtaaatga

SEQ ID NO: 50 - protein, 470 aa, Artificial Sequence
  Synthetic Construct
MGWSCIIFFLVATATGVHSQVQLVQSGAEVKKPGASVKVSCKGSGYTFTDYAMHWVRQAPGQGLEWIGVISTYYGNTNYNQKFKGRATMTVDTSTSTAYMELRSLRSDDTAVYYCARGGLREYYYAMDYWGQGTMVTVSSASTKGPSVFPLAPSSKSTSGGTAALGCLVKDYFPEPVTVSWNSGALTSGVHTFPAVLQSSGLYSLSSVVTVPSSSLGTQTYICNVNHKPSNTKVDKKVEPKSCDKTHTCPPCPAPELLGGPSVFLFPPKPKDTLMISRTPEVTCVVVDVSHEDPEVKFNWYVDGVEVHNAKTKPREEQYNSTYRVVSVLTVLHQDWLNGKEYKCKVSNKALPAPIEKTISKAKGQPREPQVYTLPPSRDELTKNQVSLTCLVKGFYPSDIAVEWESNGQPENNYKTTPPVLDSDGSFFLYSKLTVDKSRWQQGNVFSCSVMHEALHNHYTQKSLSLSPGK

SEQ ID NO: 51 - DNA, 1356 bp, Artificial Sequence
  antibody
  CDS (1)..(1356)
caagtccagctggtgcagtctggggctgaagtgaagaagcctggggcctcagtgaaagtctcctgcaagggttccggctacacattcactgattatgctatgcactgggtgcgacaggcccctggacaaggcctggagtggattggagttattagtacttactatggtaatacaaactacaaccagaagtttaagggccgagccacaatgactgtcgacacatccaccagcacagcctatatggaacttaggagcttgagatctgacgatactgccgtgtattactgtgcaagaggaggattgcgagagtattactatgctatggactactggggtcaaggaaccatggtcaccgtctcctcagcctccaccaagggcccatcggtcttccccctggcaccctcctccaagagcacctctgggggcacagcggccctgggctgcctggtcaaggactacttccccgaaccggtgacggtgtcgtggaactcaggcgccctgaccagcggcgtgcacaccttcccggctgtcctacagtcctcaggactctactccctcagcagcgtggtgaccgtgccctccagcagcttgggcacccagacctacatctgcaacgtgaatcacaagcccagcaacaccaaggtggacaagaaagttgagcccaaatcttgtgacaaaactcacacatgcccaccgtgcccagcacctgaactcctggggggaccgtcagtcttcctcttccccccaaaacccaaggacaccctcatgatctcccggacccctgaggtcacatgcgtggtggtggacgtgagccacgaagaccctgaggtcaagttcaactggtacgtggacggcgtggaggtgcataatgccaagacaaagccgcgggaggagcagtacaacagcacgtaccgtgtggtcagcgtcctcaccgtcctgcaccaggactggctgaatggcaaggagtacaagtgcaaggtctccaacaaagccctcccagcccccatcgagaaaaccatctccaaagccaaagggcagccccgagaaccacaggtgtacaccctgcccccatcccgggatgagctgaccaagaaccaggtcagcctgacctgcctggtcaaaggcttctatcccagcgacatcgccgtggagtgggagagcaatgggcagccggagaacaactacaagaccacgcctcccgtgctggactccgacggctccttcttcctctacagcaagctcaccgtggacaagagcaggtggcagcaggggaacgtcttctcatgctccgtgatgcatgaggctctgcacaaccactacacgcagaagagcctctccctgtctccgggtaaatga

SEQ ID NO: 52 - protein, 451 aa, Artificial Sequence
  Synthetic Construct
QVQLVQSGAEVKKPGASVKVSCKGSGYTFTDYAMHWVRQAPGQGLEWIGVISTYYGNTNYNQKFKGRATMTVDTSTSTAYMELRSLRSDDTAVYYCARGGLREYYYAMDYWGQGTMVTVSSASTKGPSVFPLAPSSKSTSGGTAALGCLVKDYFPEPVTVSWNSGALTSGVHTFPAVLQSSGLYSLSSVVTVPSSSLGTQTYICNVNHKPSNTKVDKKVEPKSCDKTHTCPPCPAPELLGGPSVFLFPPKPKDTLMISRTPEVTCVVVDVSHEDPEVKFNWYVDGVEVHNAKTKPREEQYNSTYRVVSVLTVLHQDWLNGKEYKCKVSNKALPAPIEKTISKAKGQPREPQVYTLPPSRDELTKNQVSLTCLVKGFYPSDIAVEWESNGQPENNYKTTPPVLDSDGSFFLYSKLTVDKSRWQQGNVFSCSVMHEALHNHYTQKSLSLSPGK

SEQ ID NO: 53 - DNA, 1413 bp, Artificial Sequence
  antibody
  CDS (1)..(1413)
atgggttggagctgtatcatcttctttctggtagcaacagctacaggcgtgcactcccaagtccagctggtgcagtctggggctgaagtgaagaagcctggggcctcagtgaaagtctcctgcaaggcttccggctacacattcactgattatgctatgcactgggtgcgacaggcccctggacaaggcctggagtggattggagttattagtacttactatggtaatacaaactacaaccagaagtttaagggcaaggccacaatgactgtcgacaaatccaccagcacagcctatatggaacttaggagcttgagatctgacgatactgccgtgtattactgtgcaagaggaggattgcgagagtattactatgctatggactactggggtcaaggaaccatggtcaccgtctcctcagcctccaccaagggcccatcggtcttccccctggcaccctcctccaagagcacctctgggggcacagcggccctgggctgcctggtcaaggactacttccccgaaccggtgacggtgtcgtggaactcaggcgccctgaccagcggcgtgcacaccttcccggctgtcctacagtcctcaggactctactccctcagcagcgtggtgaccgtgccctccagcagcttgggcacccagacctacatctgcaacgtgaatcacaagcccagcaacaccaaggtggacaagaaagttgagcccaaatcttgtgacaaaactcacacatgcccaccgtgcccagcacctgaactcctggggggaccgtcagtcttcctcttccccccaaaacccaaggacaccctcatgatctcccggacccctgaggtcacatgcgtggtggtggacgtgagccacgaagaccctgaggtcaagttcaactggtacgtggacggcgtggaggtgcataatgccaagacaaagccgcgggaggagcagtacaacagcacgtaccgtgtggtcagcgtcctcaccgtcctgcaccaggactggctgaatggcaaggagtacaagtgcaaggtctccaacaaagccctcccagcccccatcgagaaaaccatctccaaagccaaagggcagccccgagaaccacaggtgtacaccctgcccccatcccgggatgagctgaccaagaaccaggtcagcctgacctgcctggtcaaaggcttctatcccagcgacatcgccgtggagtgggagagcaatgggcagccggagaacaactacaagaccacgcctcccgtgctggactccgacggctccttcttcctctacagcaagctcaccgtggacaagagcaggtggcagcaggggaacgtcttctcatgctccgtgatgcatgaggctctgcacaaccactacacgcagaagagcctctccctgtctccgggtaaatga

SEQ ID NO: 54 - protein, 470 aa, Artificial Sequence
  Synthetic Construct
MGWSCIIFFLVATATGVHSQVQLVQSGAEVKKPGASVKVSCKASGYTFTDYAMHWVRQAPGQGLEWIGVISTYYGNTNYNQKFKGKATMTVDKSTSTAYMELRSLRSDDTAVYYCARGGLREYYYAMDYWGQGTMVTVSSASTKGPSVFPLAPSSKSTSGGTAALGCLVKDYFPEPVTVSWNSGALTSGVHTFPAVLQSSGLYSLSSVVTVPSSSLGTQTYICNVNHKPSNTKVDKKVEPKSCDKTHTCPPCPAPELLGGPSVFLFPPKPKDTLMISRTPEVTCVVVDVSHEDPEVKFNWYVDGVEVHNAKTKPREEQYNSTYRVVSVLTVLHQDWLNGKEYKCKVSNKALPAPIEKTISKAKGQPREPQVYTLPPSRDELTKNQVSLTCLVKGFYPSDIAVEWESNGQPENNYKTTPPVLDSDGSFFLYSKLTVDKSRWQQGNVFSCSVMHEALHNHYTQKSLSLSPGK

SEQ ID NO: 55 - DNA, 1356 bp, Artificial Sequence
  antibody
  CDS (1)..(1356)
caagtccagctggtgcagtctggggctgaagtgaagaagcctggggcctcagtgaaagtctcctgcaaggcttccggctacacattcactgattatgctatgcactgggtgcgacaggcccctggacaaggcctggagtggattggagttattagtacttactatggtaatacaaactacaaccagaagtttaagggcaaggccacaatgactgtcgacaaatccaccagcacagcctatatggaacttaggagcttgagatctgacgatactgccgtgtattactgtgcaagaggaggattgcgagagtattactatgctatggactactggggtcaaggaaccatggtcaccgtctcctcagcctccaccaagggcccatcggtcttccccctggcaccctcctccaagagcacctctgggggcacagcggccctgggctgcctggtcaaggactacttccccgaaccggtgacggtgtcgtggaactcaggcgccctgaccagcggcgtgcacaccttcccggctgtcctacagtcctcaggactctactccctcagcagcgtggtgaccgtgccctccagcagcttgggcacccagacctacatctgcaacgtgaatcacaagcccagcaacaccaaggtggacaagaaagttgagcccaaatcttgtgacaaaactcacacatgcccaccgtgcccagcacctgaactcctggggggaccgtcagtcttcctcttccccccaaaacccaaggacaccctcatgatctcccggacccctgaggtcacatgcgtggtggtggacgtgagccacgaagaccctgaggtcaagttcaactggtacgtggacggcgtggaggtgcataatgccaagacaaagccgcgggaggagcagtacaacagcacgtaccgtgtggtcagcgtcctcaccgtcctgcaccaggactggctgaatggcaaggagtacaagtgcaaggtctccaacaaagccctcccagcccccatcgagaaaaccatctccaaagccaaagggcagccccgagaaccacaggtgtacaccctgcccccatcccgggatgagctgaccaagaaccaggtcagcctgacctgcctggtcaaaggcttctatcccagcgacatcgccgtggagtgggagagcaatgggcagccggagaacaactacaagaccacgcctcccgtgctggactccgacggctccttcttcctctacagcaagctcaccgtggacaagagcaggtggcagcaggggaacgtcttctcatgctccgtgatgcatgaggctctgcacaaccactacacgcagaagagcctctccctgtctccgggtaaatga

SEQ ID NO: 56 - protein, 451 aa, Artificial Sequence
  Synthetic Construct
QVQLVQSGAEVKKPGASVKVSCKASGYTFTDYAMHWVRQAPGQGLEWIGVISTYYGNTNYNQKFKGKATMTVDKSTSTAYMELRSLRSDDTAVYYCARGGLREYYYAMDYWGQGTMVTVSSASTKGPSVFPLAPSSKSTSGGTAALGCLVKDYFPEPVTVSWNSGALTSGVHTFPAVLQSSGLYSLSSVVTVPSSSLGTQTYICNVNHKPSNTKVDKKVEPKSCDKTHTCPPCPAPELLGGPSVFLFPPKPKDTLMISRTPEVTCVVVDVSHEDPEVKFNWYVDGVEVHNAKTKPREEQYNSTYRVVSVLTVLHQDWLNGKEYKCKVSNKALPAPIEKTISKAKGQPREPQVYTLPPSRDELTKNQVSLTCLVKGFYPSDIAVEWESNGQPENNYKTTPPVLDSDGSFFLYSKLTVDKSRWQQGNVFSCSVMHEALHNHYTQKSLSLSPGK

SEQ ID NO: 57 - DNA, 1413 bp, Artificial Sequence
  antibody
  CDS (1)..(1413)
atgggttggagctgtatcatcttctttctggtagcaacagctacaggcgtgcactcccaagtccagctggtgcagtctggggctgaagtgaagaagcctggggcctcagtgaaagtctcctgcaaggcttccggctacacattcactgattatgctatgcactgggtgcgacaggcccctggacaaggcctggagtggattggagttattagtacttactatggtaatacaaactacaaccagaagtttaagggccgagccacaatgactgtcgacaaatccaccagcacagcctatatggaacttaggagcttgagatctgacgatactgccgtgtattactgtgcaagaggaggattgcgagagtattactatgctatggactactggggtcaaggaaccatggtcaccgtctcctcagcctccaccaagggcccatcggtcttccccctggcaccctcctccaagagcacctctgggggcacagcggccctgggctgcctggtcaaggactacttccccgaaccggtgacggtgtcgtggaactcaggcgccctgaccagcggcgtgcacaccttcccggctgtcctacagtcctcaggactctactccctcagcagcgtggtgaccgtgccctccagcagcttgggcacccagacctacatctgcaacgtgaatcacaagcccagcaacaccaaggtggacaagaaagttgagcccaaatcttgtgacaaaactcacacatgcccaccgtgcccagcacctgaactcctggggggaccgtcagtcttcctcttccccccaaaacccaaggacaccctcatgatctcccggacccctgaggtcacatgcgtggtggtggacgtgagccacgaagaccctgaggtcaagttcaactggtacgtggacggcgtggaggtgcataatgccaagacaaagccgcgggaggagcagtacaacagcacgtaccgtgtggtcagcgtcctcaccgtcctgcaccaggactggctgaatggcaaggagtacaagtgcaaggtctccaacaaagccctcccagcccccatcgagaaaaccatctccaaagccaaagggcagccccgagaaccacaggtgtacaccctgcccccatcccgggatgagctgaccaagaaccaggtcagcctgacctgcctggtcaaaggcttctatcccagcgacatcgccgtggagtgggagagcaatgggcagccggagaacaactacaagaccacgcctcccgtgctggactccgacggctccttcttcctctacagcaagctcaccgtggacaagagcaggtggcagcaggggaacgtcttctcatgctccgtgatgcatgaggctctgcacaaccactacacgcagaagagcctctccctgtctccgggtaaatga

SEQ ID NO: 58 - protein, 470 aa, Artificial Sequence
  Synthetic Construct
MGWSCIIFFLVATATGVHSQVQLVQSGAEVKKPGASVKVSCKASGYTFTDYAMHWVRQAPGQGLEWIGVISTYYGNTNYNQKFKGRATMTVDKSTSTAYMELRSLRSDDTAVYYCARGGLREYYYAMDYWGQGTMVTVSSASTKGPSVFPLAPSSKSTSGGTAALGCLVKDYFPEPVTVSWNSGALTSGVHTFPAVLQSSGLYSLSSVVTVPSSSLGTQTYICNVNHKPSNTKVDKKVEPKSCDKTHTCPPCPAPELLGGPSVFLFPPKPKDTLMISRTPEVTCVVVDVSHEDPEVKFNWYVDGVEVHNAKTKPREEQYNSTYRVVSVLTVLHQDWLNGKEYKCKVSNKALPAPIEKTISKAKGQPREPQVYTLPPSRDELTKNQVSLTCLVKGFYPSDIAVEWESNGQPENNYKTTPPVLDSDGSFFLYSKLTVDKSRWQQGNVFSCSVMHEALHNHYTQKSLSLSPGK

SEQ ID NO: 59 - DNA, 1356 bp, Artificial Sequence
  antibody
  CDS (1)..(1356)
caagtccagctggtgcagtctggggctgaagtgaagaagcctggggcctcagtgaaagtctcctgcaaggcttccggctacacattcactgattatgctatgcactgggtgcgacaggcccctggacaaggcctggagtggattggagttattagtacttactatggtaatacaaactacaaccagaagtttaagggccgagccacaatgactgtcgacaaatccaccagcacagcctatatggaacttaggagcttgagatctgacgatactgccgtgtattactgtgcaagaggaggattgcgagagtattactatgctatggactactggggtcaaggaaccatggtcaccgtctcctcagcctccaccaagggcccatcggtcttccccctggcaccctcctccaagagcacctctgggggcacagcggccctgggctgcctggtcaaggactacttccccgaaccggtgacggtgtcgtggaactcaggcgccctgaccagcggcgtgcacaccttcccggctgtcctacagtcctcaggactctactccctcagcagcgtggtgaccgtgccctccagcagcttgggcacccagacctacatctgcaacgtgaatcacaagcccagcaacaccaaggtggacaagaaagttgagcccaaatcttgtgacaaaactcacacatgcccaccgtgcccagcacctgaactcctggggggaccgtcagtcttcctcttccccccaaaacccaaggacaccctcatgatctcccggacccctgaggtcacatgcgtggtggtggacgtgagccacgaagaccctgaggtcaagttcaactggtacgtggacggcgtggaggtgcataatgccaagacaaagccgcgggaggagcagtacaacagcacgtaccgtgtggtcagcgtcctcaccgtcctgcaccaggactggctgaatggcaaggagtacaagtgcaaggtctccaacaaagccctcccagcccccatcgagaaaaccatctccaaagccaaagggcagccccgagaaccacaggtgtacaccctgcccccatcccgggatgagctgaccaagaaccaggtcagcctgacctgcctggtcaaaggcttctatcccagcgacatcgccgtggagtgggagagcaatgggcagccggagaacaactacaagaccacgcctcccgtgctggactccgacggctccttcttcctctacagcaagctcaccgtggacaagagcaggtggcagcaggggaacgtcttctcatgctccgtgatgcatgaggctctgcacaaccactacacgcagaagagcctctccctgtctccgggtaaatga

SEQ ID NO: 60 - protein, 451 aa, Artificial Sequence
  Synthetic Construct
QVQLVQSGAEVKKPGASVKVSCKASGYTFTDYAMHWVRQAPGQGLEWIGVISTYYGNTNYNQKFKGRATMTVDKSTSTAYMELRSLRSDDTAVYYCARGGLREYYYAMDYWGQGTMVTVSSASTKGPSVFPLAPSSKSTSGGTAALGCLVKDYFPEPVTVSWNSGALTSGVHTFPAVLQSSGLYSLSSVVTVPSSSLGTQTYICNVNHKPSNTKVDKKVEPKSCDKTHTCPPCPAPELLGGPSVFLFPPKPKDTLMISRTPEVTCVVVDVSHEDPEVKFNWYVDGVEVHNAKTKPREEQYNSTYRVVSVLTVLHQDWLNGKEYKCKVSNKALPAPIEKTISKAKGQPREPQVYTLPPSRDELTKNQVSLTCLVKGFYPSDIAVEWESNGQPENNYKTTPPVLDSDGSFFLYSKLTVDKSRWQQGNVFSCSVMHEALHNHYTQKSLSLSPGK

SEQ ID NO: 61 - DNA, 1413 bp, Artificial Sequence
  antibody
  CDS (1)..(1413)
atgggttggagctgtatcatcttctttctggtagcaacagctacaggcgtgcactcccaagtccagctggtgcagtctggggctgaagtgaagaagcctggggcctcagtgaaagtctcctgcaagggttccggctacacattcactgattatgctatgcactgggtgcgacaggcccctggacaaggcctggagtggattggagttattagtacttactatggtaatacaaactacaaccagaagtttaagggcaaggccacaatgactgtcgacaaatccaccagcacagcctatatggaacttaggagcttgagatctgacgatactgccgtgtattactgtgcaagaggaggattgcgagagtattactatgctatggactactggggtcaaggaaccatggtcaccgtctcctcagcctccaccaagggcccatcggtcttccccctggcaccctcctccaagagcacctctgggggcacagcggccctgggctgcctggtcaaggactacttccccgaaccggtgacggtgtcgtggaactcaggcgccctgaccagcggcgtgcacaccttcccggctgtcctacagtcctcaggactctactccctcagcagcgtggtgaccgtgccctccagcagcttgggcacccagacctacatctgcaacgtgaatcacaagcccagcaacaccaaggtggacaagaaagttgagcccaaatcttgtgacaaaactcacacatgcccaccgtgcccagcacctgaactcctggggggaccgtcagtcttcctcttccccccaaaacccaaggacaccctcatgatctcccggacccctgaggtcacatgcgtggtggtggacgtgagccacgaagaccctgaggtcaagttcaactggtacgtggacggcgtggaggtgcataatgccaagacaaagccgcgggaggagcagtacaacagcacgtaccgtgtggtcagcgtcctcaccgtcctgcaccaggactggctgaatggcaaggagtacaagtgcaaggtctccaacaaagccctcccagcccccatcgagaaaaccatctccaaagccaaagggcagccccgagaaccacaggtgtacaccctgcccccatcccgggatgagctgaccaagaaccaggtcagcctgacctgcctggtcaaaggcttctatcccagcgacatcgccgtggagtgggagagcaatgggcagccggagaacaactacaagaccacgcctcccgtgctggactccgacggctccttcttcctctacagcaagctcaccgtggacaagagcaggtggcagcaggggaacgtcttctcatgctccgtgatgcatgaggctctgcacaaccactacacgcagaagagcctctccctgtctccgggtaaatga

SEQ ID NO: 62 - protein, 470 aa, Artificial Sequence
  Synthetic Construct
MGWSCIIFFLVATATGVHSQVQLVQSGAEVKKPGASVKVSCKGSGYTFTDYAMHWVRQAPGQGLEWIGVISTYYGNTNYNQKFKGKATMTVDKSTSTAYMELRSLRSDDTAVYYCARGGLREYYYAMDYWGQGTMVTVSSASTKGPSVFPLAPSSKSTSGGTAALGCLVKDYFPEPVTVSWNSGALTSGVHTFPAVLQSSGLYSLSSVVTVPSSSLGTQTYICNVNHKPSNTKVDKKVEPKSCDKTHTCPPCPAPELLGGPSVFLFPPKPKDTLMISRTPEVTCVVVDVSHEDPEVKFNWYVDGVEVHNAKTKPREEQYNSTYRVVSVLTVLHQDWLNGKEYKCKVSNKALPAPIEKTISKAKGQPREPQVYTLPPSRDELTKNQVSLTCLVKGFYPSDIAVEWESNGQPENNYKTTPPVLDSDGSFFLYSKLTVDKSRWQQGNVFSCSVMHEALHNHYTQKSLSLSPGK

SEQ ID NO: 63 - DNA, 1356 bp, Artificial Sequence
  antibody
  CDS (1)..(1356)
caagtccagctggtgcagtctggggctgaagtgaagaagcctggggcctcagtgaaagtctcctgcaagggttccggctacacattcactgattatgctatgcactgggtgcgacaggcccctggacaaggcctggagtggattggagttattagtacttactatggtaatacaaactacaaccagaagtttaagggcaaggccacaatgactgtcgacaaatccaccagcacagcctatatggaacttaggagcttgagatctgacgatactgccgtgtattactgtgcaagaggaggattgcgagagtattactatgctatggactactggggtcaaggaaccatggtcaccgtctcctcagcctccaccaagggcccatcggtcttccccctggcaccctcctccaagagcacctctgggggcacagcggccctgggctgcctggtcaaggactacttccccgaaccggtgacggtgtcgtggaactcaggcgccctgaccagcggcgtgcacaccttcccggctgtcctacagtcctcaggactctactccctcagcagcgtggtgaccgtgccctccagcagcttgggcacccagacctacatctgcaacgtgaatcacaagcccagcaacaccaaggtggacaagaaagttgagcccaaatcttgtgacaaaactcacacatgcccaccgtgcccagcacctgaactcctggggggaccgtcagtcttcctcttccccccaaaacccaaggacaccctcatgatctcccggacccctgaggtcacatgcgtggtggtggacgtgagccacgaagaccctgaggtcaagttcaactggtacgtggacggcgtggaggtgcataatgccaagacaaagccgcgggaggagcagtacaacagcacgtaccgtgtggtcagcgtcctcaccgtcctgcaccaggactggctgaatggcaaggagtacaagtgcaaggtctccaacaaagccctcccagcccccatcgagaaaaccatctccaaagccaaagggcagccccgagaaccacaggtgtacaccctgcccccatcccgggatgagctgaccaagaaccaggtcagcctgacctgcctggtcaaaggcttctatcccagcgacatcgccgtggagtgggagagcaatgggcagccggagaacaactacaagaccacgcctcccgtgctggactccgacggctccttcttcctctacagcaagctcaccgtggacaagagcaggtggcagcaggggaacgtcttctcatgctccgtgatgcatgaggctctgcacaaccactacacgcagaagagcctctccctgtctccgggtaaatga

SEQ ID NO: 64 - protein, 451 aa, Artificial Sequence
  Synthetic Construct
QVQLVQSGAEVKKPGASVKVSCKGSGYTFTDYAMHWVRQAPGQGLEWIGVISTYYGNTNYNQKFKGKATMTVDKSTSTAYMELRSLRSDDTAVYYCARGGLREYYYAMDYWGQGTMVTVSSASTKGPSVFPLAPSSKSTSGGTAALGCLVKDYFPEPVTVSWNSGALTSGVHTFPAVLQSSGLYSLSSVVTVPSSSLGTQTYICNVNHKPSNTKVDKKVEPKSCDKTHTCPPCPAPELLGGPSVFLFPPKPKDTLMISRTPEVTCVVVDVSHEDPEVKFNWYVDGVEVHNAKTKPREEQYNSTYRVVSVLTVLHQDWLNGKEYKCKVSNKALPAPIEKTISKAKGQPREPQVYTLPPSRDELTKNQVSLTCLVKGFYPSDIAVEWESNGQPENNYKTTPPVLDSDGSFFLYSKLTVDKSRWQQGNVFSCSVMHEALHNHYTQKSLSLSPGK

SEQ ID NO: 65 - DNA, 1413 bp, Artificial Sequence
  antibody
  CDS (1)..(1413)
atgggttggagctgtatcatcttctttctggtagcaacagctacaggcgtgcactcccaagtccagctggtgcagtctggggctgaagtgaagaagcctggggcctcagtgaaagtctcctgcaagggttccggctacacattcactgattatgctatgcactgggtgcgacaggcccctggacaaggcctggagtggattggagttattagtacttactatggtaatacaaactacaaccagaagtttaagggccgagccacaatgactgtcgacaaatccaccagcacagcctatatggaacttaggagcttgagatctgacgatactgccgtgtattactgtgcaagaggaggattgcgagagtattactatgctatggactactggggtcaaggaaccatggtcaccgtctcctcagcctccaccaagggcccatcggtcttccccctggcaccctcctccaagagcacctctgggggcacagcggccctgggctgcctggtcaaggactacttccccgaaccggtgacggtgtcgtggaactcaggcgccctgaccagcggcgtgcacaccttcccggctgtcctacagtcctcaggactctactccctcagcagcgtggtgaccgtgccctccagcagcttgggcacccagacctacatctgcaacgtgaatcacaagcccagcaacaccaaggtggacaagaaagttgagcccaaatcttgtgacaaaactcacacatgcccaccgtgcccagcacctgaactcctggggggaccgtcagtcttcctcttccccccaaaacccaaggacaccctcatgatctcccggacccctgaggtcacatgcgtggtggtggacgtgagccacgaagaccctgaggtcaagttcaactggtacgtggacggcgtggaggtgcataatgccaagacaaagccgcgggaggagcagtacaacagcacgtaccgtgtggtcagcgtcctcaccgtcctgcaccaggactggctgaatggcaaggagtacaagtgcaaggtctccaacaaagccctcccagcccccatcgagaaaaccatctccaaagccaaagggcagccccgagaaccacaggtgtacaccctgcccccatcccgggatgagctgaccaagaaccaggtcagcctgacctgcctggtcaaaggcttctatcccagcgacatcgccgtggagtgggagagcaatgggcagccggagaacaactacaagaccacgcctcccgtgctggactccgacggctccttcttcctctacagcaagctcaccgtggacaagagcaggtggcagcaggggaacgtcttctcatgctccgtgatgcatgaggctctgcacaaccactacacgcagaagagcctctccctgtctccgggtaaatga

SEQ ID NO: 66 - protein, 470 aa, Artificial Sequence
  Synthetic Construct
MGWSCIIFFLVATATGVHSQVQLVQSGAEVKKPGASVKVSCKGSGYTFTDYAMHWVRQAPGQGLEWIGVISTYYGNTNYNQKFKGRATMTVDKSTSTAYMELRSLRSDDTAVYYCARGGLREYYYAMDYWGQGTMVTVSSASTKGPSVFPLAPSSKSTSGGTAALGCLVKDYFPEPVTVSWNSGALTSGVHTFPAVLQSSGLYSLSSVVTVPSSSLGTQTYICNVNHKPSNTKVDKKVEPKSCDKTHTCPPCPAPELLGGPSVFLFPPKPKDTLMISRTPEVTCVVVDVSHEDPEVKFNWYVDGVEVHNAKTKPREEQYNSTYRVVSVLTVLHQDWLNGKEYKCKVSNKALPAPIEKTISKAKGQPREPQVYTLPPSRDELTKNQVSLTCLVKGFYPSDIAVEWESNGQPENNYKTTPPVLDSDGSFFLYSKLTVDKSRWQQGNVFSCSVMHEALHNHYTQKSLSLSPGK

SEQ ID NO: 67 - DNA, 1356 bp, Artificial Sequence
  antibody
  CDS (1)..(1356)
caagtccagctggtgcagtctggggctgaagtgaagaagcctggggcctcagtgaaagtctcctgcaagggttccggctacacattcactgattatgctatgcactgggtgcgacaggcccctggacaaggcctggagtggattggagttattagtacttactatggtaatacaaactacaaccagaagtttaagggccgagccacaatgactgtcgacaaatccaccagcacagcctatatggaacttaggagcttgagatctgacgatactgccgtgtattactgtgcaagaggaggattgcgagagtattactatgctatggactactggggtcaaggaaccatggtcaccgtctcctcagcctccaccaagggcccatcggtcttccccctggcaccctcctccaagagcacctctgggggcacagcggccctgggctgcctggtcaaggactacttccccgaaccggtgacggtgtcgtggaactcaggcgccctgaccagcggcgtgcacaccttcccggctgtcctacagtcctcaggactctactccctcagcagcgtggtgaccgtgccctccagcagcttgggcacccagacctacatctgcaacgtgaatcacaagcccagcaacaccaaggtggacaagaaagttgagcccaaatcttgtgacaaaactcacacatgcccaccgtgcccagcacctgaactcctggggggaccgtcagtcttcctcttccccccaaaacccaaggacaccctcatgatctcccggacccctgaggtcacatgcgtggtggtggacgtgagccacgaagaccctgaggtcaagttcaactggtacgtggacggcgtggaggtgcataatgccaagacaaagccgcgggaggagcagtacaacagcacgtaccgtgtggtcagcgtcctcaccgtcctgcaccaggactggctgaatggcaaggagtacaagtgcaaggtctccaacaaagccctcccagcccccatcgagaaaaccatctccaaagccaaagggcagccccgagaaccacaggtgtacaccctgcccccatcccgggatgagctgaccaagaaccaggtcagcctgacctgcctggtcaaaggcttctatcccagcgacatcgccgtggagtgggagagcaatgggcagccggagaacaactacaagaccacgcctcccgtgctggactccgacggctccttcttcctctacagcaagctcaccgtggacaagagcaggtggcagcaggggaacgtcttctcatgctccgtgatgcatgaggctctgcacaaccactacacgcagaagagcctctccctgtctccgggtaaatga

SEQ ID NO: 68 - protein, 451 aa, Artificial Sequence
  Synthetic Construct
QVQLVQSGAEVKKPGASVKVSCKGSGYTFTDYAMHWVRQAPGQGLEWIGVISTYYGNTNYNQKFKGRATMTVDKSTSTAYMELRSLRSDDTAVYYCARGGLREYYYAMDYWGQGTMVTVSSASTKGPSVFPLAPSSKSTSGGTAALGCLVKDYFPEPVTVSWNSGALTSGVHTFPAVLQSSGLYSLSSVVTVPSSSLGTQTYICNVNHKPSNTKVDKKVEPKSCDKTHTCPPCPAPELLGGPSVFLFPPKPKDTLMISRTPEVTCVVVDVSHEDPEVKFNWYVDGVEVHNAKTKPREEQYNSTYRVVSVLTVLHQDWLNGKEYKCKVSNKALPAPIEKTISKAKGQPREPQVYTLPPSRDELTKNQVSLTCLVKGFYPSDIAVEWESNGQPENNYKTTPPVLDSDGSFFLYSKLTVDKSRWQQGNVFSCSVMHEALHNHYTQKSLSLSPGK

SEQ ID NO: 69 - DNA, 723 bp, Artificial Sequence
  antibody
  CDS (1)..(723)
atggaatcacagacccaggtcctcatgtttcttctgctctgggtatctggtgcctgtgcagacattgtcatgacacagtctccagactccctggctgtgtcactgggagagagggccactatcaactgcaagtccagtcagagccttctgaatagtagcaatcaaaagaactatttggcctggtaccagcagaaaccaggacagcctcctaaacttctggtctactttgcatccactagggaatctggggtccctgatcgcttcagtggcagtggatctgggacagatttcactcttaccatcagcagtctgcaggctgaagatgtggcagtttactactgtcagcaacattatagcactcctcccacattcggtcaggggaccaagctggagatcaaacgaactgtggctgcaccatctgtcttcatcttcccgccatctgatgagcagttgaaatctggaactgcctctgttgtgtgcctgctgaataacttctatcccagagaggccaaagtacagtggaaggtggataacgccctccaatcgggtaactcccaggagagtgtcacagagcaggacagcaaggacagcacctacagcctcagcagcaccctgacgctgagcaaagcagactacgagaaacacaaagtctacgcctgcgaagtcacccatcagggcctgagctcgcccgtcacaaagagcttcaacaggggagagtgttag

SEQ ID NO: 70 - protein, 240 aa, Artificial Sequence
  Synthetic Construct
MESQTQVLMFLLLWVSGACADIVMTQSPDSLAVSLGERATINCKSSQSLLNSSNQKNYLAWYQQKPGQPPKLLVYFASTRESGVPDRFSGSGSGTDFTLTISSLQAEDVAVYYCQQHYSTPPTFGQGTKLEIKRTVAAPSVFIFPPSDEQLKSGTASVVCLLNNFYPREAKVQWKVDNALQSGNSQESVTEQDSKDSTYSLSSTLTLSKADYEKHKVYACEVTHQGLSSPVTKSFNRGEC

SEQ ID NO: 71 - DNA, 663 bp, Artificial Sequence
  antibody
  CDS (1)..(663)
gacattgtcatgacacagtctccagactccctggctgtgtcactgggagagagggccactatcaactgcaagtccagtcagagccttctgaatagtagcaatcaaaagaactatttggcctggtaccagcagaaaccaggacagcctcctaaacttctggtctactttgcatccactagggaatctggggtccctgatcgcttcagtggcagtggatctgggacagatttcactcttaccatcagcagtctgcaggctgaagatgtggcagtttactactgtcagcaacattatagcactcctcccacattcggtcaggggaccaagctggagatcaaacgaactgtggctgcaccatctgtcttcatcttcccgccatctgatgagcagttgaaatctggaactgcctctgttgtgtgcctgctgaataacttctatcccagagaggccaaagtacagtggaaggtggataacgccctccaatcgggtaactcccaggagagtgtcacagagcaggacagcaaggacagcacctacagcctcagcagcaccctgacgctgagcaaagcagactacgagaaacacaaagtctacgcctgcgaagtcacccatcagggcctgagctcgcccgtcacaaagagcttcaacaggggagagtgttag

SEQ ID NO: 72 - protein, 220 aa, Artificial Sequence
  Synthetic Construct
DIVMTQSPDSLAVSLGERATINCKSSQSLLNSSNQKNYLAWYQQKPGQPPKLLVYFASTRESGVPDRFSGSGSGTDFTLTISSLQAEDVAVYYCQQHYSTPPTFGQGTKLEIKRTVAAPSVFIFPPSDEQLKSGTASVVCLLNNFYPREAKVQWKVDNALQSGNSQESVTEQDSKDSTYSLSSTLTLSKADYEKHKVYACEVTHQGLSSPVTKSFNRGEC

SEQ ID NO: 73 - protein, 5 aa, Artificial Sequence
  CDRH1
DYAMH

SEQ ID NO: 74 - protein, 17 aa, Artificial Sequence
  CDRH2
VISTYYGNTNYNQKFKG

SEQ ID NO: 75 - protein, 12 aa, Artificial Sequence
  CDRH3
GGLREYYYAMDY

SEQ ID NO: 76 - protein, 17 aa, Artificial Sequence
  CDRL1
KSSQSLLNSSNQKNYLA

SEQ ID NO: 77 - protein, 7 aa, Artificial Sequence
  CDRL2
FASTRES

SEQ ID NO: 78 - protein, 9 aa, Artificial Sequence
  CDRL3
QQHYSTPPT